European Patent Application EP 4 549 470 A1, published May 7, 2025. Title: Peptide and associate or composition including the peptide. Applicant: MeSCue-Janusys Inc. Application JP. The sequence listing filed with the application follows.

SEQUENCE LISTING (20 sequences)

SEQ ID NO: 1 - protein, 20 aa, synthetic construct
  REGION 1..20: note = a peptide designed to have two hydrophilic regions and a hydrophobic region located therebetween
  MOD_RES 3: note = PHOSPHORYLATION
  MOD_RES 18: note = ACETYLATION
DSSEEKWLLELLELLRRKRR

SEQ ID NO: 2 - protein, 20 aa, synthetic construct
  REGION 1..20: note = a peptide designed to have two hydrophilic regions and a hydrophobic region located therebetween
  MOD_RES 3: note = PHOSPHORYLATION
DSSEEKWLLELLELLRRKRR

SEQ ID NO: 3 - protein, 19 aa, synthetic construct
  REGION 1..19: note = a peptide designed to have two hydrophilic regions and a hydrophobic region located therebetween
  MOD_RES 3: note = PHOSPHORYLATION
  MOD_RES 17: note = ACETYLATION
DSSEEKWWEWWEWWRRKRR

SEQ ID NO: 4 - protein, 19 aa, synthetic construct
  REGION 1..19: note = a peptide designed to have two hydrophilic regions and a hydrophobic region located therebetween
  MOD_RES 3: note = PHOSPHORYLATION
  MOD_RES 17: note = ACETYLATION
DSSEEKAAEAAEAARRKRR

SEQ ID NO: 5 - protein, 23 aa, synthetic construct
  REGION 1..23: note = a peptide designed to have two hydrophilic regions and a hydrophobic region located therebetween
  MOD_RES 3: note = PHOSPHORYLATION
DSSEEKWLLELLELLKGKILRPR

SEQ ID NO: 6 - protein, 24 aa, synthetic construct
  REGION 1..24: note = a peptide designed to have two hydrophilic regions and a hydrophobic region located therebetween
GRSHHKRKLLELLELLHRHHVQER

SEQ ID NO: 7 - protein, 24 aa, synthetic construct
  REGION 1..24: note = a peptide designed to have two hydrophilic regions and a hydrophobic region located therebetween
HHIRRKRQWWEWWEWWHGDHHKSN

SEQ ID NO: 8 - protein, 16 aa, synthetic construct
  REGION 1..16: note = a peptide designed to have a hydrophilic region and a hydrophobic region
KGKILRPRLLLLLLLL

SEQ ID NO: 9 - protein, 16 aa, synthetic construct
  REGION 1..16: note = a peptide designed to have a hydrophilic region and a hydrophobic region
KGKILRPRYYYYYYYY

SEQ ID NO: 10 - protein, 16 aa, synthetic construct
  REGION 1..16: note = a peptide designed to have a hydrophilic region and a hydrophobic region
KGKILRPRWWWWWWWW

SEQ ID NO: 11 - protein, 16 aa, synthetic construct
  REGION 1..16: note = a peptide designed to have a hydrophilic region and a hydrophobic region
KGKILRPRFFFFFFFF

SEQ ID NO: 12 - protein, 16 aa, synthetic construct
  REGION 1..16: note = a peptide designed to have a hydrophilic region and a hydrophobic region
KGKILRPRLLELLELL

SEQ ID NO: 13 - protein, 16 aa, synthetic construct
  REGION 1..16: note = a peptide designed to have a hydrophilic region and a hydrophobic region
KGKILRPRWWEWWEWW

SEQ ID NO: 14 - protein, 16 aa, synthetic construct
  REGION 1..16: note = a peptide designed to have a hydrophilic region and a hydrophobic region
KGKILRPRAAEAAEAA

SEQ ID NO: 15 - protein, 16 aa, synthetic construct
  REGION 1..16: note = a peptide designed to have a hydrophilic region and a hydrophobic region
KGKILRPRAAAAAAAA

SEQ ID NO: 16 - protein, 5 aa, synthetic construct
  REGION 1..5: note = Rgp-binding peptide
RRKRR

SEQ ID NO: 17 - protein, 7 aa, synthetic construct
  REGION 1..7: note = HA-binding peptide
  MOD_RES 3: note = PHOSPHORYLATION
DSSEEKW

SEQ ID NO: 18 - protein, 10 aa, synthetic construct
GYSEWRKWEL

SEQ ID NO: 19 - protein, 16 aa, synthetic construct
GYSEWRKWELLLLLLL

SEQ ID NO: 20 - protein, 24 aa, synthetic construct
GYSEWRKWELLLLLLLGGHWRGWV